European Patent Application EP 4 253 405 A2, published October 4, 2023. Title: Variant of BPIFB4 Protein. Applicant: LGV1 S.R.L. The sequence listing filed with the application follows.

SEQUENCE LISTING (11 sequences)

SEQ ID NO: 1 - protein, 575 aa, Homo sapiens
MLQQSDALHSALREVPLGVGDIPYNDFHVRGPPPVYTNGKKLDGIYQYGHIETNDNTAQLGGKYRYGEILESEGSIRDLRNSGYRSAENAYGGHRGLGRYRAAPVGRLHRRELQPGEIPPGVATGAVGPGGLLGTGGMLAADGILAGQGGLLGGGGLLGDGGLLGGGGVLGVLGEGGILSTVQGITGLRIVELTLPRVSVRLLPGVGVYLSLYTRVAINGKSLIGFLDVAVEVNITAKVRLTMDRTGYPRLVIERCDTLLGGIKVKLLRGLLPNLVDNLVTRVLADVLPDLLCPIVDVVLGLVNDQLGLVDSLIPLGILGSVQYTFSSLPLVTGEFLELDLNTLVGEAGGGLIDYPLGWPAVSPKPMPELPPMGDNTKSQLAMSANFLGSVLTLLQKQHALDLDITNGMFEELPPLTTATLGALIPKVFQQYPESCPLIIRIQVLNPPSVMLQKDKALVKVLATAEVMVSQPKDLETTICLIDVDTEFLASFSTEGDKLMIDAKLEKTSLNLRTSNVGNFDIGLMEVLVEKIFDLAFMPAMNAVLGSGVPLPKILNIDFSNADIDVLEDLLVLSA

SEQ ID NO: 2 - DNA, 1728 bp, Homo sapiens
  source 1..1728: mol_type = unassigned DNA
atgctgcagcaaagtgatgctctccactcggccctgagagaggtgcccttgggtgttggtgatattccctacaatgacttccatgtccgaggaccccccccagtatataccaacggcaaaaaacttgatggtatttaccagtatggtcacattgagaccaacgacaacactgctcagctggggggcaaataccgatatggtgagatccttgagtccgagggaagcatcagggacctccgaaacagtggctatcgcagtgccgagaatgcatatggaggccacaggggcctcgggcgatacagggcagcacctgtgggcaggcttcaccggcgagagctgcagcctggagaaatcccacctggagttgccactggggcggtgggcccaggtggtttgctgggcactggaggcatgctggcagctgatggcatcctcgcaggccaaggtggcctgctcggcggaggtggtctccttggtgatggaggacttcttggaggagggggtgtcctgggcgtgctcggcgagggtggcatcctcagcactgtgcaaggcatcacggggctgcgtatcgtggagctgaccctccctcgggtgtccgtgcggctcctgcccggcgtgggtgtctacctgagcttgtacacccgtgtggccatcaacgggaagagtcttattggcttcctggacgtcgcagtagaagtgaacatcacagccaaggtccggctgaccatggaccgcacgggttatcctcggctggtcattgagcgatgtgacaccctcctagggggcatcaaagtcaagctgctgcgagggcttctccccaatctcgtggacaatttagtgacccgagtcctggccgacgtcctccctgacttgctctgccccatcgtggatgtggtgctgggtcttgtcaatgaccagctgggcctcgtggattctctgattcctctggggatattgggaagtgtccagtacaccttctccagcctcccgcttgtgaccggggaattcctggagctggacctcaacacgctggttggggaggctggaggaggactcatcgactacccattggggtggccagctgtgtctcccaagccgatgccagagctgcctcccatgggtgacaacaccaagtcccagctggccatgtctgccaacttcctgggctcagtgctgactctactgcagaagcagcatgctctagacctggatatcaccaatggcatgtttgaagagcttcctccacttaccacagccacactgggagccctgatccccaaggtgttccagcagtaccccgagtcctgcccacttatcatcaggatccaggtgctgaacccaccatctgtgatgctgcagaaggacaaagcgctggtgaaggtgttggccactgccgaggtcatggtctcccagcccaaagacctggagactaccatctgcctcattgacgtggacacagaattcttggcctcattttccacagaaggagataagctcatgattgatgccaagctggagaagaccagcctcaacctcagaacctcaaacgtgggcaactttgatattggcctcatggaggtgctggtggagaagatttttgacctggcattcatgcccgcaatgaacgctgtgctgggttctggcgtccctctccccaaaatcctcaacatcgactttagcaatgcagacattgacgtgttggaggaccttttggtgctgagcgcatga

SEQ ID NO: 3 - protein, 575 aa, Homo sapiens
MLQQSDALHSALREVPLGVGDIPYNDFHVRGPPPVYTNGKKLDGIYQYGHIETNDNTAQLGGKYRYGEILESEGSIRDLRNSGYRSAENAYGGHRGLGRYRAAPVGRLHRRELQPGEIPPGVATGAVGPGGLLGTGGMLAADGILAGQGGLLGGGGLLGDGGLLGGGGVLGVLGEGGILSTVQGITGLRIVELTLPRVSVRLLPGVGVYLSLYTRVAINGKSLIGFLDIAVEVNITAKVRLTMDRTGYPRLVIERCDTLLGGIKVKLLRGLLPNLVDNLVNRVLADVLPDLLCPIVDVVLGLVNDQLGLVDSLIPLGILGSVQYTFSSLPLVTGEFLELDLNTLVGEAGGGLIDYPLGWPAVSPKPMPELPPMGDNTKSQLAMSANFLGSVLTLLQKQHALDLDITNGMFEELPPLTTATLGALIPKVFQQYPESCPLIIRIQVLNPPSVMLQKDKALVKVLATAEVMVSQPKDLETTICLIDVDTEFLASFSTEGDKLMIDAKLEKTSLNLRTSNVGNFDIGLMEVLVEKIFDLAFMPAMNAVLGSGVPLPKILNIDFSNADIDVLEDLLVLSA

SEQ ID NO: 4 - protein, 575 aa, Homo sapiens
MLQQSDALHSALREVPLGVGDIPYNDFHVRGPPPVYTNGKKLDGIYQYGHIETNDNTAQLGGKYRYGEILESEGSIRDLRNSGYRSAENAYGGHRGLGRYRAAPVGRLHRRELQPGEIPPGVATGAVGPGGLLGTGGMLAADGILAGQGGLLGGGGLLGDGGLLGGGGVLGVLGEGGILSTVQGITGLRIVELTLPRVSVRLLPGVGVYLSLYTRVAINGKSLIGFLDVAVEVNITAKVRLTMDRTGYPRLVIERCDTLLGGIKVKLLRGLLPNLVDNLVNRVLADVLPDLLCPIVDVVLGLVNDQLGLVDSLIPLGILGSVQYTFSSLPLVTGEFLELDLNTLVGEAGGGLIDYPLGWPAVSPKPMPELPPMGDNTKSQLAMSANFLGSVLTLLQKQHALDLDITNGMFEELPPLTTATLGALIPKVFQQYPESCPLIIRIQVLNPPSVMLQKDKALVKVLATAEVMVSQPKDLETTICLIDVDTEFLASFSTEGDKLMIDAKLEKTSLNLRTSNVGNFDIGLMEVLVEKIFDLAFMPAMNAVLGSGVPLPKILNIDFSNADIDVLEDLLVLSA

SEQ ID NO: 5 - protein, 575 aa, Homo sapiens
MLQQSDALHSALREVPLGVGDIPYNDFHVRGPPPVYTNGKKLDGIYQYGHIETNDNTAQLGGKYRYGEILESEGSIRDLRNSGYRSAENAYGGHRGLGRYRAAPVGRLHRRELQPGEIPPGVATGAVGPGGLLGTGGMLAADGILAGQGGLLGGGGLLGDGGLLGGGGVLGVLGEGGILSTVQGITGLRIVELTLPRVSVRLLPGVGVYLSLYTRVAINGKSLIGFLDIAVEVNITAKVRLTMDRTGYPRLVIERCDTLLGGIKVKLLRGLLPNLVDNLVTRVLADVLPDLLCPIVDVVLGLVNDQLGLVDSLIPLGILGSVQYTFSSLPLVTGEFLELDLNTLVGEAGGGLIDYPLGWPAVSPKPMPELPPMGDNTKSQLAMSANFLGSVLTLLQKQHALDLDITNGMFEELPPLTTATLGALIPKVFQQYPESCPLIIRIQVLNPPSVMLQKDKALVKVLATAEVMVSQPKDLETTICLIDVDTEFLASFSTEGDKLMIDAKLEKTSLNLRTSNVGNFDIGLMEVLVEKIFDLAFMPAMNAVLGSGVPLPKILNIDFSNADIDVLEDLLVLSA

SEQ ID NO: 6 - protein, 575 aa, Homo sapiens
MLQQSDALHSALREVPLGVGDIPYNDFHVRGPPPVYTNGKKLDGIYQYGHIETNDNTAQLGGKYRYGEILESEGSIRDLRNSGYRSAENAYGGHRGLGRYRAAPVGRLHRRELQPGEIPPGVATGAVGPGGLLGTGGMLAADGILAGQGGLLGGGGLLGDGGLLGGGGVLGVLGEGGILSTVQGITGLRIVELTLPRVSVRLLPGVGVYLSLYTRVAINGKSLIGFLDVAVEVNITAKVRLTMDRTGYPRLVIERCDTLLGGIKVKLLRGLLPNLVDNLVTRVLADVLPDLLCPIVDVVLGLVNDQLGLVDSLIPLGILGSVQYTFSSLPLVTGEFLELDLNTLVGEAGGGLIDYPLGWPAVSPKPMPELPPMGDNTKSQLAMSANFLGSVLTLLQKQHALDLDITNGMFEELPPLTTATLGALIPKVFQQYPESCPLIIRIQVLNPPSVMLQKDKALVKVLATAEVMVSQPKDLETTICLIDVDTELLASFSIEGDKLMIDAKLEKTSLNLRTSNVGNFDIGLMEVLVEKIFDLAFMPAMNAVLGSGVPLPKILNIDFSNADIDVLEDLLVLSA

SEQ ID NO: 7 - protein, 575 aa, Homo sapiens
MLQQSDALHSALREVPLGVGDIPYNDFHVRGPPPVYTNGKKLDGIYQYGHIETNDNTAQLGGKYRYGEILESEGSIRDLRNSGYRSAENAYGGHRGLGRYRAAPVGRLHRRELQPGEIPPGVATGAVGPGGLLGTGGMLAADGILAGQGGLLGGGGLLGDGGLLGGGGVLGVLGEGGILSTVQGITGLRIVELTLPRVSVRLLPGVGVYLSLYTRVAINGKSLIGFLDIAVEVNITAKVRLTMDRTGYPRLVIERCDTLLGGIKVKLLRGLLPNLVDNLVNRVLADVLPDLLCPIVDVVLGLVNDQLGLVDSLIPLGILGSVQYTFSSLPLVTGEFLELDLNTLVGEAGGGLIDYPLGWPAVSPKPMPELPPMGDNTKSQLAMSANFLGSVLTLLQKQHALDLDITNGMFEELPPLTTATLGALIPKVFQQYPESCPLIIRIQVLNPPSVMLQKDKALVKVLATAEVMVSQPKDLETTICLIDVDTELLASFSIEGDKLMIDAKLEKTSLNLRTSNVGNFDIGLMEVLVEKIFDLAFMPAMNAVLGSGVPLPKILNIDFSNADIDVLEDLLVLSA

SEQ ID NO: 8 - DNA, 21 bp, synthetic construct
  misc_feature 1..21: note = Primer
  source 1..21: mol_type = other DNA
ctctccccaaaatcctcaaca

SEQ ID NO: 9 - DNA, 20 bp, synthetic construct
  misc_feature 1..20: note = Primer
  source 1..20: mol_type = other DNA
agcctctctgggactggttc

SEQ ID NO: 10 - DNA, 19 bp, synthetic construct
  misc_feature 1..19: note = Primer
  source 1..19: mol_type = other DNA
gtgaaggtcggagtcaacg

SEQ ID NO: 11 - DNA, 22 bp, synthetic construct
  misc_feature 1..22: note = Primer
  source 1..22: mol_type = other DNA
ggtggaatcatattggaacatg